European Patent Specification EP 3 998 288 B1, published July 30, 2025. Title: FUSION PROTEIN AND COMPOSITION FOR TREATING ANIMAL TUMORS. Applicant: BEIJING KENUOKEFU BIOTECHNOLOGY CO., LTD. The sequence listing filed with the application follows.

SEQUENCE LISTING (6 sequences)

SEQ ID NO: 1 - protein, 817 aa, Artificial Sequence
  SIGNAL (1)..(817): Fusion protein
IWELEKDVYVVELDWHPDAPGEMVVLTCHTPEEDDITWTSAQSSEVLGSGKTLTIQVKEFGDAGQYTCHKGGKVLSRSLLLIHKKEDGIWSTDILKEQKESKNKIFLKCEAKNYSGRFTCWWLTAISTDLKFSVKSSRGFSDPQGVTCGAVTLSAERVRVDNRDYKKYTVECQEGSACPSAEESLPIEVVVDAIHKLKYENYTSSFFIRDIIKPDPPTNLQLKPLKNSRHVEVSWEYPDTWSTPHSYFSLTFCVQAQGKNNREKKDRLCVDKTSAKVVCHKDAKIRVQARDRYYSSSWSDWASVSCSGGGGSGGGGSGGGGSRSLPTASPSPGIFQCLNHSQNLLRAVSNTLQKARQTLELYSCTSEEIDHEDITKDKTSTVEACLPLELTMNESCLASREISLITNGSCLASGKASFMTVLCLSSIYEDLKMYQMEFKAMNAKLLMDPKRQIFLDQNMLTAIDELLQALNFNSVTVPQKSSLEEPDFYKTKIKLCILLHAFRIRAVTIDRMMSYLNSSGGGGSGGGGSGGGGSAPITSSSTKETEQQMEQLLLDLQLLLNGVNNYENPQLSRMLTFKFYTPKKATEFTHLQCLAEELKNLEEVLGLPQSKNVHLTDTKELISNMNVTLLKLKGSETSYNCEYDDETATITEFLNKWITFCQSIFSTLTGGGGSGGGGSGGGGSAPTRSPTLVTRPSQHVDAIQEALSLLNNSNDVTAVMNKAVKVVSEVFDPEGPTCLETRLQLYKEGLQGSLTSLKNPLTMMANHYKQHCPPTPESPCATQNINFKSFKENLKDFLFNIPFDCWKPVKKHHHHHH

SEQ ID NO: 2 - protein, 817 aa, Artificial Sequence
  SIGNAL (1)..(817): Fusion protein
IWELEKDVYVVELDWHPDAPGEMVVLTCHTPEEDDITWTSAQSSEVLGSGKTLTIQVKEFGDAGQYTCHKGGKVLSRSLLLIHKKEDGIWSTDILKEQKESKNKIFLKCEAKNYSGRFTCWWLTAISTDLKFSVKSSRGFSDPQGVTCGAVTLSAERVRVDNRDYKKYTVECQEGSACPSAEESLPIEVVVDAIHKLKYENYTSSFFIRDIIKPDPPTNLQLKPLKNSRHVEVSWEYPDTWSTPHSYFSLTFCVQAQGKNNREKKDRLCVDKTSAKVVCHKDAKIRVQARDRYYSSSWSDWASVSCSGGGGSGGGGSGGGGSRSLPTASPSPGIFQCLNHSQNLLRAVSNTLQKARQTLELYSCTSEEIDHEDITKDKTSTVEACLPLELTMNESCLASREISLITNGSCLASGKASFMTVLCLSSIYEDLKMYQMEFKAMNAKLLMDPKRQIFLDQNMLTAIDELLQALNFNSVTVPQKSSLEEPDFYKTKIKLCILLHAFRIRAVTIDRMMSYLNSSGGGGSGGGGSGGGGSAPTRSPTLVTRPSQHVDAIQEALSLLNNSNDVTAVMNKAVKVVSEVFDPEGPTCLETRLQLYKEGLQGSLTSLKNPLTMMANHYKQHCPPTPESPCATQNINFKSFKENLKDFLFNIPFDCWKPVKKGGGGSGGGGSGGGGSAPITSSSTKETEQQMEQLLLDLQLLLNGVNNYENPQLSRMLTFKFYTPKKATEFTHLQCLAEELKNLEEVLGLPQSKNVHLTDTKELISNMNVTLLKLKGSETSYNCEYDDETATITEFLNKWITFCQSIFSTLTHHHHHH

SEQ ID NO: 3 - protein, 816 aa, Artificial Sequence
  SIGNAL (1)..(816): Fusion protein
IWELEKNVYVVELDWHPDAPGEMVVLTCNTPEEDDITWTSDQSSEVLGSGKTLTIQVKEFADAGQYTCHKGGEVLSHSFLLIHKKEDGIWSTDILREQKESKNKIFLKCEAKNYSGRFTCWWLTAISTDLKFTVKSSRGSSDPQEVTCGAATLSAEKVRVDNRDYKKYTVECQEGSACPAAEESLPIEVVVDAIHKLKYENYTSSFFIRDIIKPDPPKNLQLKPLKNSRHVEVSWEYPDTWSTPHSYFSLTFGVQVQGKNNREKKDRLSVDKTSAKVVCHKDAKIRVQARDRYYSSSWSNWASVSCSGGGGSGGGGSGGGGSRNLPTPTPSPGMFQCLNHSQTLLRAISNTLQKARQTLEFYPCTSEEIDHEDITKDKTSTVEACLPLELTMNESCLASREISLITNGSCLASRKTSFMTTLCLSSIYEDLKMYQVEFKAMNAKLLMDPKRQIFLDQNMLTAIDELLQALNVNSVTVPQNSSLEEPDFYKTKIKLCILLHAFRIRAVTINRMMSYLNSSGGGGSGGGGSGGGGSAPASSSTKETQQQLEQLLLDLRLLLNGVNNPENPKLSRMLTFKFYVPKKATELTHLQCLVEELKPLEEVLYLAQSKNFHLNHIKELMSNINVTVLKLKGSETRFTCNYDDETATIVEFLNKWITFCQSIFSTLTGGGGSGGGGSGGGGSAPTSSPSSVTRPWQHVDAMKEALSLLNNSSEITAVMNETVEVVSEMFDPEEPKCLQTHLKLYEQGLRGSLISLKEPLRMMANHYKQHCPLTPETPCETQTITFKNFKEKLKDFLFNNPFDCWGPDQKHHHHHH

SEQ ID NO: 4 - protein, 816 aa, Artificial Sequence
  SIGNAL (1)..(816): Fusion protein
IWELEKNVYVVELDWHPDAPGEMVVLTCNTPEEDDITWTSDQSSEVLGSGKTLTIQVKEFADAGQYTCHKGGEVLSHSFLLIHKKEDGIWSTDILREQKESKNKIFLKCEAKNYSGRFTCWWLTAISTDLKFTVKSSRGSSDPQEVTCGAATLSAEKVRVDNRDYKKYTVECQEGSACPAAEESLPIEVVVDAIHKLKYENYTSSFFIRDIIKPDPPKNLQLKPLKNSRHVEVSWEYPDTWSTPHSYFSLTFGVQVQGKNNREKKDRLSVDKTSAKVVCHKDAKIRVQARDRYYSSSWSNWASVSCSGGGGSGGGGSGGGGSRNLPTPTPSPGMFQCLNHSQTLLRAISNTLQKARQTLEFYPCTSEEIDHEDITKDKTSTVEACLPLELTMNESCLASREISLITNGSCLASRKTSFMTTLCLSSIYEDLKMYQVEFKAMNAKLLMDPKRQIFLDQNMLTAIDELLQALNVNSVTVPQNSSLEEPDFYKTKIKLCILLHAFRIRAVTINRMMSYLNSSGGGGSGGGGSGGGGSAPTSSPSSVTRPWQHVDAMKEALSLLNNSSEITAVMNETVEVVSEMFDPEEPKCLQTHLKLYEQGLRGSLISLKEPLRMMANHYKQHCPLTPETPCETQTITFKNFKEKLKDFLFNNPFDCWGPDQKGGGGSGGGGSGGGGSAPASSSTKETQQQLEQLLLDLRLLLNGVNNPENPKLSRMLTFKFYVPKKATELTHLQCLVEELKPLEEVLYLAQSKNFHLNHIKELMSNINVTVLKLKGSETRFTCNYDDETATIVEFLNKWITFCQSIFSTLTHHHHHH

SEQ ID NO: 5 - protein, 1309 aa, Artificial Sequence
  SIGNAL (1)..(1309): Fusion protein
IWELEKDVYVVELDWHPDAPGEMVVLTCHTPEEDDITWTSAQSSEVLGSGKTLTIQVKEFGDAGQYTCHKGGKVLSRSLLLIHKKEDGIWSTDILKEQKESKNKIFLKCEAKNYSGRFTCWWLTAISTDLKFSVKSSRGFSDPQGVTCGAVTLSAERVRVDNRDYKKYTVECQEGSACPSAEESLPIEVVVDAIHKLKYENYTSSFFIRDIIKPDPPTNLQLKPLKNSRHVEVSWEYPDTWSTPHSYFSLTFCVQAQGKNNREKKDRLCVDKTSAKVVCHKDAKIRVQARDRYYSSSWSDWASVSCSGGGGSGGGGSGGGGSRSLPTASPSPGIFQCLNHSQNLLRAVSNTLQKARQTLELYSCTSEEIDHEDITKDKTSTVEACLPLELTMNESCLASREISLITNGSCLASGKASFMTVLCLSSIYEDLKMYQMEFKAMNAKLLMDPKRQIFLDQNMLTAIDELLQALNFNSVTVPQKSSLEEPDFYKTKIKLCILLHAFRIRAVTIDRMMSYLNSSGGGGSGGGGSGGGGSAPITSSSTKETEQQMEQLLLDLQLLLNGVNNYENPQLSRMLTFKFYTPKKATEFTHLQCLAEELKNLEEVLGLPQSKNVHLTDTKELISNMNVTLLKLKGSETSYNCEYDDETATITEFLNKWITFCQSIFSTLTGGGGSLVPRGSGGGGSQVQLQESGPGLVKPSETLSLTCAVSGYSISSGYYWGWIRQPPGKGLEWIGSIYHSGSTYYNPSLKSRVTISVDTSKNQFSLKLSSVTAADTAVYYCARGKWSKFDYWGQGTLVTVSSGGSGGEIVLTQSPGTLSLSPGERATLSCRASQSVSMPFLAWYQQKPGQAPRLLIYGASSRATGIPDRFSGSGSGTDFTLTISRLEPEDFAVYYCQQMRGRPPTFGQGTKVEIKSSSSGSSSSGSSSSGEVQLLESGGGLVQPGGSLRLSCAASGFTFSLFTMSWVRQAPGKGLEWVSAISGSGGSTYYADSVKGRFTISRDNSKNTLYLQMNSLRAEDTAVYYCAKSTHLYLFDYWGQGTLVTVSSGGSGGSSELTQDPAVSVALGQTVRITCQGDSLRSYYASWYQQKPGQAPVLVIYGKNNRPSGIPDRFSGSSSGNTASLTITGAQAEDEADYYCNSRDSSGNHVVFGGGTKLTVLSSSSGLVPRGSSSSGAPTRSPTLVTRPSQHVDAIQEALSLLNNSNDVTAVMNKAVKVVSEVFDPEGPTCLETRLQLYKEGLQGSLTSLKNPLTMMANHYKQHCPPTPESPCATQNINFKSFKENLKDFLFNIPFDCWKPVKKHHHHHH

SEQ ID NO: 6 - protein, 1308 aa, Artificial Sequence
  SIGNAL (1)..(1308): Fusion protein
IWELEKNVYVVELDWHPDAPGEMVVLTCNTPEEDDITWTSDQSSEVLGSGKTLTIQVKEFADAGQYTCHKGGEVLSHSFLLIHKKEDGIWSTDILREQKESKNKIFLKCEAKNYSGRFTCWWLTAISTDLKFTVKSSRGSSDPQEVTCGAATLSAEKVRVDNRDYKKYTVECQEGSACPAAEESLPIEVVVDAIHKLKYENYTSSFFIRDIIKPDPPKNLQLKPLKNSRHVEVSWEYPDTWSTPHSYFSLTFGVQVQGKNNREKKDRLSVDKTSAKVVCHKDAKIRVQARDRYYSSSWSNWASVSCSGGGGSGGGGSGGGGSRNLPTPTPSPGMFQCLNHSQTLLRAISNTLQKARQTLEFYPCTSEEIDHEDITKDKTSTVEACLPLELTMNESCLASREISLITNGSCLASRKTSFMTTLCLSSIYEDLKMYQVEFKAMNAKLLMDPKRQIFLDQNMLTAIDELLQALNVNSVTVPQNSSLEEPDFYKTKIKLCILLHAFRIRAVTINRMMSYLNSSGGGGSGGGGSGGGGSAPASSSTKETQQQLEQLLLDLRLLLNGVNNPENPKLSRMLTFKFYVPKKATELTHLQCLVEELKPLEEVLYLAQSKNFHLNHIKELMSNINVTVLKLKGSETRFTCNYDDETATIVEFLNKWITFCQSIFSTLTGGGGSLVPRGSGGGGSQVQLQESGPGLVKPSETLSLTCAVSGYSISSGYYWGWIRQPPGKGLEWIGSIYHSGSTYYNPSLKSRVTISVDTSKNQFSLKLSSVTAADTAVYYCARGKWSKFDYWGQGTLVTVSSGGSGGEIVLTQSPGTLSLSPGERATLSCRASQSVSMPFLAWYQQKPGQAPRLLIYGASSRATGIPDRFSGSGSGTDFTLTISRLEPEDFAVYYCQQMRGRPPTFGQGTKVEIKSSSSGSSSSGSSSSGEVQLLESGGGLVQPGGSLRLSCAASGFTFSLFTMSWVRQAPGKGLEWVSAISGSGGSTYYADSVKGRFTISRDNSKNTLYLQMNSLRAEDTAVYYCAKSTHLYLFDYWGQGTLVTVSSGGSGGSSELTQDPAVSVALGQTVRITCQGDSLRSYYASWYQQKPGQAPVLVIYGKNNRPSGIPDRFSGSSSGNTASLTITGAQAEDEADYYCNSRDSSGNHVVFGGGTKLTVLSSSSGLVPRGSSSSGAPTSSPSSVTRPWQHVDAMKEALSLLNNSSEITAVMNETVEVVSEMFDPEEPKCLQTHLKLYEQGLRGSLISLKEPLRMMANHYKQHCPLTPETPCETQTITFKNFKEKLKDFLFNNPFDCWGPDQKHHHHHH